European Patent Specification EP 3 705 498 B1, published February 25, 2026. Title: TGF-BETA RECEPTOR TYPE II VARIANTS AND USES THEREOF. Applicant: KUMAR, RAVINDRA GRINBERG, ASYA SAKO, DIANNE S. CASTONGUAY, ROSELYNE STEEVES, RITA. Application PCT/US2014/052130. The sequence listing filed with the application follows.

SEQUENCE LISTING (69 sequences)

SEQ ID NO: 1 - protein, 308 aa, Homo sapiens
MPGQELRTVNGSQMLLVLLVLSWLPHGGALSLAEASRASFPGPSELHSEDSRFRELRKRYEDLLTRLRANQSWEDSNTDLVPAPAVRILTPEVRLGSGGHLHLRISRAALPEGLPEASRLHRALFRLSPTASRSWDVTRPLRRQLSLARPQAPALHLRLSPPPSQSDQLLAESSSARPQLELHLRPQAARGRRRARARNGDHCPLGPGRCCRLHTVRASLEDLGWADWVLSPREVQVTMCIGACPSQFRAANMHAQIKTSLHRLKPDTVPAPCCVPASYNPMVLIQKTDTGVSLQTYDDLLAKDCHCI

SEQ ID NO: 2 - DNA, 924 bp, Homo sapiens
atgcccgggcaagaactcaggacggtgaatggctctcagatgctcctggtgttgctggtgctctcgtggctgccgcatgggggcgccctgtctctggccgaggcgagccgcgcaagtttcccgggaccctcagagttgcactccgaagactccagattccgagagttgcggaaacgctacgaggacctgctaaccaggctgcgggccaaccagagctgggaagattcgaacaccgacctcgtcccggcccctgcagtccggatactcacgccagaagtgcggctgggatccggcggccacctgcacctgcgtatctctcgggccgcccttcccgaggggctccccgaggcctcccgccttcaccgggctctgttccggctgtccccgacggcgtcaaggtcgtgggacgtgacacgaccgctgcggcgtcagctcagccttgcaagaccccaggcacccgcgctgcacctgcgactgtcgccgccgccgtcgcagtcggaccaactgctggcagaatcttcgtccgcacggccccagctggagttgcacttgcggccgcaagccgccagggggcgccgcagagcgcgtgcgcgcaacggggaccactgtccgctcgggcccgggcgttgctgccgtctgcacacggtccgcgcgtcgctggaagacctgggctgggccgattgggtgctgtcgccacgggaggtgcaagtgaccatgtgcatcggcgcgtgcccgagccagttccgggcggcaaacatgcacgcgcagatcaagacgagcctgcaccgcctgaagcccgacacggtgccagcgccctgctgcgtgcccgccagctacaatcccatggtgctcattcaaaagaccgacaccggggtgtcactccagacctatgatgacttgttagccaaagactgccactgcata

SEQ ID NO: 3 - protein, 303 aa, Mus musculus
MAPPALQAQPPGGSQLRFLLFLLLLLLLLSWPSQGDALAMPEQRPSGPESQLNADELRGRFQDLLSRLHANQSREDSNSEPSPDPAVRILSPEVRLGSHGQLLLRVNRASLSQGLPEAYRVHRALLLLTPTARPWDITRPLKRALSLRGPRAPALRLRLTPPPDLAMLPSGGTQLELRLRVAAGRGRRSAHAHPRDSCPLGPGRCCHLETVQATLEDLGWSDWVLSPRQLQLSMCVGECPHLYRSANTHAQIKARLHGLQPDKVPAPCCVPSSYTPVVLMHRTDSGVSLQTYDDLVARGCHCA

SEQ ID NO: 4 - DNA, 909 bp, Mus musculus
atggccccgcccgcgctccaggcccagcctccaggcggctctcaactgaggttcctgctgttcctgctgctgttgctgctgctgctgtcatggccatcgcagggggacgccctggcaatgcctgaacagcgaccctccggccctgagtcccaactcaacgccgacgagctacggggtcgcttccaggacctgctgagccggctgcatgccaaccagagccgagaggactcgaactcagaaccaagtcctgacccagctgtccggatactcagtccagaggtgagattggggtcccacggccagctgctactccgcgtcaaccgggcgtcgctgagtcagggtctccccgaagcctaccgcgtgcaccgagcgctgctcctgctgacgccgacggcccgcccctgggacatcactaggcccctgaagcgtgcgctcagcctccggggaccccgtgctcccgcattacgcctgcgcctgacgccgcctccggacctggctatgctgccctctggcggcacgcagctggaactgcgcttacgggtagccgccggcagggggcgccgaagcgcgcatgcgcacccaagagactcgtgcccactgggtccagggcgctgctgtcacttggagactgtgcaggcaactcttgaagacttgggctggagcgactgggtgctgtccccgcgccagctgcagctgagcatgtgcgtgggcgagtgtccccacctgtatcgctccgcgaacacgcatgcgcagatcaaagcacgcctgcatggcctgcagcctgacaaggtgcctgccccgtgctgtgtcccctccagctacaccccggtggttcttatgcacaggacagacagtggtgtgtcactgcagacttatgatgacctggtggcccggggctgccactgcgct

SEQ ID NO: 5 - protein, 567 aa, Homo sapiens
MGRGLLRGLWPLHIVLWTRIASTIPPHVQKSVNNDMIVTDNNGAVKFPQLCKFCDVRFSTCDNQKSCMSNCSITSICEKPQEVCVAVWRKNDENITLETVCHDPKLPYHDFILEDAASPKCIMKEKKKPGETFFMCSCSSDECNDNIIFSEEYNTSNPDLLLVIFQVTGISLLPPLGVAISVIIIFYCYRVNRQQKLSSTWETGKTRKLMEFSEHCAIILEDDRSDISSTCANNINHNTELLPIELDTLVGKGRFAEVYKAKLKQNTSEQFETVAVKIFPYEEYASWKTEKDIFSDINLKHENILQFLTAEERKTELGKQYWLITAFHAKGNLQEYLTRHVISWEDLRKLGSSLARGIAHLHSDHTPCGRPKMPIVHRDLKSSNILVKNDLTCCLCDFGLSLRLDPTLSVDDLANSGQVGTARYMAPEVLESRMNLENVESFKQTDVYSMALVLWEMTSRCNAVGEVKDYEPPFGSKVREHPCVESMKDNVLRDRGRPEIPSFWLNHQGIQMVCETLTECWDHDPEARLTAQCVAERFSELEHLDRLSGRSCSEEKIPEDGSLNTTK

SEQ ID NO: 6 - protein, 592 aa, Homo sapiens
MGRGLLRGLWPLHIVLWTRIASTIPPHVQKSDVEMEAQKDEIICPSCNRTAHPLRHINNDMIVTDNNGAVKFPQLCKFCDVRFSTCDNQKSCMSNCSITSICEKPQEVCVAVWRKNDENITLETVCHDPKLPYHDFILEDAASPKCIMKEKKKPGETFFMCSCSSDECNDNIIFSEEYNTSNPDLLLVIFQVTGISLLPPLGVAISVIIIFYCYRVNRQQKLSSTWETGKTRKLMEFSEHCAIILEDDRSDISSTCANNINHNTELLPIELDTLVGKGRFAEVYKAKLKQNTSEQFETVAVKIFPYEEYASWKTEKDIFSDINLKHENILQFLTAEERKTELGKQYWLITAFHAKGNLQEYLTRHVISWEDLRKLGSSLARGIAHLHSDHTPCGRPKMPIVHRDLKSSNILVKNDLTCCLCDFGLSLRLDPTLSVDDLANSGQVGTARYMAPEVLESRMNLENVESFKQTDVYSMALVLWEMTSRCNAVGEVKDYEPPFGSKVREHPCVESMKDNVLRDRGRPEIPSFWLNHQGIQMVCETLTECWDHDPEARLTAQCVAERFSELEHLDRLSGRSCSEEKIPEDGSLNTTK

SEQ ID NO: 7 - protein, 137 aa, Homo sapiens
TIPPHVQKSVNNDMIVTDNNGAVKFPQLCKFCDVRFSTCDNQKSCMSNCSITSICEKPQEVCVAVWRKNDENITLETVCHDPKLPYHDFILEDAASPKCIMKEKKKPGETFFMCSCSSDECNDNIIFSEEYNTSNPD

SEQ ID NO: 8 - protein, 137 aa, Artificial Sequence
  Description of Artificial Sequence: Synthetic polypeptide
TIPPHVQKSVNNDMIVTDNNGAVKFPQLCKFCDVRFSTCDNQKSCMSNCSITSICEKPQEVCVAVWRKNDENITLETVCHDPKLPYHKFILEDAASPKCIMKEKKKPGETFFMCSCSSDECNDNIIFSEEYNTSNPD

SEQ ID NO: 9 - protein, 131 aa, Artificial Sequence
  Description of Artificial Sequence: Synthetic polypeptide
QKSVNNDMIVTDNNGAVKFPQLCKFCDVRFSTCDNQKSCMSNCSITSICEKPQEVCVAVWRKNDENITLETVCHDPKLPYHDFILEDAASPKCIMKEKKKPGETFFMCSCSSDECNDNIIFSEEYNTSNPD

SEQ ID NO: 10 - protein, 125 aa, Artificial Sequence
  Description of Artificial Sequence: Synthetic polypeptide
DMIVTDNNGAVKFPQLCKFCDVRFSTCDNQKSCMSNCSITSICEKPQEVCVAVWRKNDENITLETVCHDPKLPYHDFILEDAASPKCIMKEKKKPGETFFMCSCSSDECNDNIIFSEEYNTSNPD

SEQ ID NO: 11 - protein, 131 aa, Artificial Sequence
  Description of Artificial Sequence: Synthetic polypeptide
TIPPHVQKSVNNDMIVTDNNGAVKFPQLCKFCDVRFSTCDNQKSCMSNCSITSICEKPQEVCVAVWRKNDENITLETVCHDPKLPYHDFILEDAASPKCIMKEKKKPGETFFMCSCSSDECNDNIIFSEEY

SEQ ID NO: 12 - protein, 131 aa, Artificial Sequence
  Description of Artificial Sequence: Synthetic polypeptide
TIPPHVQKSVNNDMIVTDNNGAVKFPQLCKFCDVRFSTCDNQKSCMSDCSITSICEKPQEVCVAVWRKNDENITLETVCHDPKLPYHDFILEDAASPKCIMKEKKKPGETFFMCSCSSDECNDNIIFSEEY

SEQ ID NO: 13 - protein, 162 aa, Artificial Sequence
  Description of Artificial Sequence: Synthetic polypeptide
TIPPHVQKSDVEMEAQKDEIICPSCNRTAHPLRHINNDMIVTDNNGAVKFPQLCKFCDVRFSTCDNQKSCMSNCSITSICEKPQEVCVAVWRKNDENITLETVCHDPKLPYHDFILEDAASPKCIMKEKKKPGETFFMCSCSSDECNDNIIFSEEYNTSNPD

SEQ ID NO: 14 - protein, 162 aa, Artificial Sequence
  Description of Artificial Sequence: Synthetic polypeptide
TIPPHVQKSDVEMEAQKDEIICPSCNRTAHPLRHINNDMIVTDNNGAVKFPQLCKFCDVRFSTCDNQKSCMSNCSITSICEKPQEVCVAVWRKNDENITLETVCHDPKLPYHKFILEDAASPKCIMKEKKKPGETFFMCSCSSDECNDNIIFSEEYNTSNPD

SEQ ID NO: 15 - protein, 156 aa, Artificial Sequence
  Description of Artificial Sequence: Synthetic polypeptide
QKSDVEMEAQKDEIICPSCNRTAHPLRHINNDMIVTDNNGAVKFPQLCKFCDVRFSTCDNQKSCMSNCSITSICEKPQEVCVAVWRKNDENITLETVCHDPKLPYHDFILEDAASPKCIMKEKKKPGETFFMCSCSSDECNDNIIFSEEYNTSNPD

SEQ ID NO: 16 - protein, 156 aa, Artificial Sequence
  Description of Artificial Sequence: Synthetic polypeptide
TIPPHVQKSDVEMEAQKDEIICPSCNRTAHPLRHINNDMIVTDNNGAVKFPQLCKFCDVRFSTCDNQKSCMSNCSITSICEKPQEVCVAVWRKNDENITLETVCHDPKLPYHDFILEDAASPKCIMKEKKKPGETFFMCSCSSDECNDNIIFSEEY

SEQ ID NO: 17 - protein, 156 aa, Artificial Sequence
  Description of Artificial Sequence: Synthetic polypeptide
TIPPHVQKSDVEMEAQKDEIICPSCNRTAHPLRHINNDMIVTDNNGAVKFPQLCKFCDVRFSTCDNQKSCMSDCSITSICEKPQEVCVAVWRKNDENITLETVCHDPKLPYHDFILEDAASPKCIMKEKKKPGETFFMCSCSSDECNDNIIFSEEY

SEQ ID NO: 18 - protein, 36 aa, Homo sapiens
GRCKIRHIGSNNRLQRSTCQNTGWESAHVMKTPGFR

SEQ ID NO: 19 - protein, 223 aa, Homo sapiens
VECPPCPAPPVAGPSVFLFPPKPKDTLMISRTPEVTCVVVDVSHEDPEVQFNWYVDGVEVHNAKTKPREEQFNSTFRVVSVLTVVHQDWLNGKEYKCKVSNKGLPAPIEKTISKTKGQPREPQVYTLPPSREEMTKNQVSLTCLVKGFYPSDIAVEWESNGQPENNYKTTPPMLDSDGSFFLYSKLTVDKSRWQQGNVFSCSVMHEALHNHYTQKSLSLSPGK

SEQ ID NO: 20 - protein, 233 aa, Homo sapiens
GGPKSCDKTHTCPPCPAPELLGGPSVFLFPPKPKDTLMISRTPEVTCVVVDVSHEDPEVKFNWYVDGVEVHNAKTKPREEQYNSTYRVVSVLTVLHQDWLNGKEYKCKVSNKALPAPIEKTISKAKGQPREPQVYTLPPSREEMTKNQVSLTCLVKGFYPSDIAVEWESNGQPENNYKTTPPVLDSDGSFFLYSKLTVDKSRWQQGNVFSCSVMHEALHNHYTQKSLSLSPGK

SEQ ID NO: 21 - protein, 225 aa, Homo sapiens
THTCPPCPAPELLGGPSVFLFPPKPKDTLMISRTPEVTCVVVDVSHEDPEVKFNWYVDGVEVHNAKTKPREEQYNSTYRVVSVLTVLHQDWLNGKEYKCKVSNKALPAPIEKTISKAKGQPREPQVYTLPPSREEMTKNQVSLTCLVKGFYPSDIAVEWESNGQPENNYKTTPPVLDSDGSFFLYSKLTVDKSRWQQGNVFSCSVMHEALHNHYTQKSLSLSPGK

SEQ ID NO: 22 - protein, 22 aa, Unknown
  Description of Unknown: Native leader peptide sequence
MGRGLLRGLWPLHIVLWTRIAS

SEQ ID NO: 23 - protein, 22 aa, Unknown
  Description of Unknown: Tissue plasminogen activator (TPA) leader peptide sequence
MDAMKRGLCCVLLLCGAVFVSP

SEQ ID NO: 24 - protein, 21 aa, Apis mellifera
MKFLVNVALVFMVVYISYIYA

SEQ ID NO: 25 - protein, 388 aa, Artificial Sequence
  Description of Artificial Sequence: Synthetic polypeptide
MDAMKRGLCCVLLLCGAVFVSPGATIPPHVQKSVNNDMIVTDNNGAVKFPQLCKFCDVRFSTCDNQKSCMSNCSITSICEKPQEVCVAVWRKNDENITLETVCHDPKLPYHKFILEDAASPKCIMKEKKKPGETFFMCSCSSDECNDNIIFSEEYNTSNPDTGGGVECPPCPAPPVAGPSVFLFPPKPKDTLMISRTPEVTCVVVDVSHEDPEVQFNWYVDGVEVHNAKTKPREEQFNSTFRVVSVLTVVHQDWLNGKEYKCKVSNKGLPAPIEKTISKTKGQPREPQVYTLPPSREEMTKNQVSLTCLVKGFYPSDIAVEWESNGQPENNYKTTPPMLDSDGSFFLYSKLTVDKSRWQQGNVFSCSVMHEALHNHYTQKSLSLSPGK

SEQ ID NO: 26 - DNA, 1164 bp, Artificial Sequence
  Description of Artificial Sequence: Synthetic polynucleotide
atggatgcaatgaagagagggctctgctgtgtgctgctgctgtgtggagcagtcttcgtttcgcccggcgccacgatcccaccgcacgttcagaagtcggttaataacgacatgatagtcactgacaacaacggtgcagtcaagtttccacaactgtgtaaattttgtgatgtgagattttccacctgtgacaaccagaaatcctgcatgagcaactgcagcatcacctccatctgtgagaagccacaggaagtctgtgtggctgtatggagaaagaatgacgagaacataacactagagacagtttgccatgaccccaagctcccctaccataagtttattctggaagatgctgcttctccaaagtgcattatgaaggaaaaaaaaaagcctggtgagactttcttcatgtgttcctgtagctctgatgagtgcaatgacaacatcatcttctcagaagaatataacaccagcaatcctgacaccggtggtggagtcgagtgcccaccgtgcccagcaccacctgtggcaggaccgtcagtcttcctcttccccccaaaacccaaggacaccctcatgatctcccggacccctgaggtcacgtgcgtggtggtggacgtgagccacgaagaccccgaggtccagttcaactggtacgtggacggcgtggaggtgcataatgccaagacaaagccacgggaggagcagttcaacagcacgttccgtgtggtcagcgtcctcaccgtcgtgcaccaggactggctgaacggcaaggagtacaagtgcaaggtctccaacaaaggcctcccagcccccatcgagaaaaccatctccaaaaccaaagggcagccccgagaaccacaggtgtacaccctgcccccatcccgggaggagatgaccaagaaccaggtcagcctgacctgcctggtcaaaggcttctaccccagcgacatcgccgtggagtgggagagcaatgggcagccggagaacaactacaagaccacacctcccatgctggactccgacggctccttcttcctctacagcaagctcaccgtggacaagagcaggtggcagcaggggaacgtcttctcatgctccgtgatgcatgaggctctgcacaaccactacacgcagaagagcctctccctgtctccgggtaaa

SEQ ID NO: 27 - protein, 390 aa, Artificial Sequence
  Description of Artificial Sequence: Synthetic polypeptide
MDAMKRGLCCVLLLCGAVFVSPGATIPPHVQKSVNNDMIVTDNNGAVKFPQLCKFCDVRFSTCDNQKSCMSNCSITSICEKPQEVCVAVWRKNDENITLETVCHDPKLPYHKFILEDAASPKCIMKEKKKPGETFFMCSCSSDECNDNIIFSEEYNTSNPDTGGGTHTCPPCPAPELLGGPSVFLFPPKPKDTLMISRTPEVTCVVVDVSHEDPEVKFNWYVDGVEVHNAKTKPREEQYNSTYRVVSVLTVLHQDWLNGKEYKCKVSNKALPAPIEKTISKAKGQPREPQVYTLPPSREEMTKNQVSLTCLVKGFYPSDIAVEWESNGQPENNYKTTPPVLDSDGSFFLYSKLTVDKSRWQQGNVFSCSVMHEALHNHYTQKSLSLSPGK

SEQ ID NO: 28 - DNA, 1170 bp, Artificial Sequence
  Description of Artificial Sequence: Synthetic polynucleotide
atggatgcaatgaagagagggctctgctgtgtgctgctgctgtgtggagcagtcttcgtttcgcccggcgccacgatcccaccgcacgttcagaagtcggttaataacgacatgatagtcactgacaacaacggtgcagtcaagtttccacaactgtgtaaattttgtgatgtgagattttccacctgtgacaaccagaaatcctgcatgagcaactgcagcatcacctccatctgtgagaagccacaggaagtctgtgtggctgtatggagaaagaatgacgagaacataacactagagacagtttgccatgaccccaagctcccctaccataagtttattctggaagatgctgcttctccaaagtgcattatgaaggaaaaaaaaaagcctggtgagactttcttcatgtgttcctgtagctctgatgagtgcaatgacaacatcatcttctcagaagaatataacaccagcaatcctgacaccggtggtggaactcacacatgcccaccgtgcccagcacctgaactcctggggggaccgtcagtcttcctcttccccccaaaacccaaggacaccctcatgatctcccggacccctgaggtcacatgcgtggtggtggacgtgagccacgaagaccctgaggtcaagttcaactggtacgtggacggcgtggaggtgcataatgccaagacaaagccgcgggaggagcagtacaacagcacgtaccgtgtggtcagcgtcctcaccgtcctgcaccaggactggctgaatggcaaggagtacaagtgcaaggtctccaacaaagccctcccagcccccatcgagaaaaccatctccaaagccaaagggcagccccgagaaccacaggtgtacaccctgcccccatcccgggaggagatgaccaagaaccaggtcagcctgacctgcctggtcaaaggcttctatcccagcgacatcgccgtggagtgggagagcaatgggcagccggagaacaactacaagaccacgcctcccgtgctggactccgacggctccttcttcctctatagcaagctcaccgtggacaagagcaggtggcagcaggggaacgtcttctcatgctccgtgatgcatgaggctctgcacaaccactacacgcagaagagcctctccctgtccccgggtaaa

SEQ ID NO: 29 - protein, 382 aa, Artificial Sequence
  Description of Artificial Sequence: Synthetic polypeptide
MDAMKRGLCCVLLLCGAVFVSPGAQKSVNNDMIVTDNNGAVKFPQLCKFCDVRFSTCDNQKSCMSNCSITSICEKPQEVCVAVWRKNDENITLETVCHDPKLPYHDFILEDAASPKCIMKEKKKPGETFFMCSCSSDECNDNIIFSEEYNTSNPDTGGGVECPPCPAPPVAGPSVFLFPPKPKDTLMISRTPEVTCVVVDVSHEDPEVQFNWYVDGVEVHNAKTKPREEQFNSTFRVVSVLTVVHQDWLNGKEYKCKVSNKGLPAPIEKTISKTKGQPREPQVYTLPPSREEMTKNQVSLTCLVKGFYPSDIAVEWESNGQPENNYKTTPPMLDSDGSFFLYSKLTVDKSRWQQGNVFSCSVMHEALHNHYTQKSLSLSPGK

SEQ ID NO: 30 - DNA, 1146 bp, Artificial Sequence
  Description of Artificial Sequence: Synthetic polynucleotide
atggatgcaatgaagagagggctctgctgtgtgctgctgctgtgtggagcagtcttcgtttcgcccggcgcccagaagtcggttaataacgacatgatagtcactgacaacaacggtgcagtcaagtttccacaactgtgtaaattttgtgatgtgagattttccacctgtgacaaccagaaatcctgcatgagcaactgcagcatcacctccatctgtgagaagccacaggaagtctgtgtggctgtatggagaaagaatgacgagaacataacactagagacagtttgccatgaccccaagctcccctaccatgactttattctggaagatgctgcttctccaaagtgcattatgaaggaaaaaaaaaagcctggtgagactttcttcatgtgttcctgtagctctgatgagtgcaatgacaacatcatcttctcagaagaatataacaccagcaatcctgacaccggtggtggagtcgagtgcccaccgtgcccagcaccacctgtggcaggaccgtcagtcttcctcttccccccaaaacccaaggacaccctcatgatctcccggacccctgaggtcacgtgcgtggtggtggacgtgagccacgaagaccccgaggtccagttcaactggtacgtggacggcgtggaggtgcataatgccaagacaaagccacgggaggagcagttcaacagcacgttccgtgtggtcagcgtcctcaccgtcgtgcaccaggactggctgaacggcaaggagtacaagtgcaaggtctccaacaaaggcctcccagcccccatcgagaaaaccatctccaaaaccaaagggcagccccgagaaccacaggtgtacaccctgcccccatcccgggaggagatgaccaagaaccaggtcagcctgacctgcctggtcaaaggcttctaccccagcgacatcgccgtggagtgggagagcaatgggcagccggagaacaactacaagaccacacctcccatgctggactccgacggctccttcttcctctacagcaagctcaccgtggacaagagcaggtggcagcaggggaacgtcttctcatgctccgtgatgcatgaggctctgcacaaccactacacgcagaagagcctctccctgtctccgggtaaa

SEQ ID NO: 31 - protein, 384 aa, Artificial Sequence
  Description of Artificial Sequence: Synthetic polypeptide
MDAMKRGLCCVLLLCGAVFVSPGAQKSVNNDMIVTDNNGAVKFPQLCKFCDVRFSTCDNQKSCMSNCSITSICEKPQEVCVAVWRKNDENITLETVCHDPKLPYHDFILEDAASPKCIMKEKKKPGETFFMCSCSSDECNDNIIFSEEYNTSNPDTGGGTHTCPPCPAPELLGGPSVFLFPPKPKDTLMISRTPEVTCVVVDVSHEDPEVKFNWYVDGVEVHNAKTKPREEQYNSTYRVVSVLTVLHQDWLNGKEYKCKVSNKALPAPIEKTISKAKGQPREPQVYTLPPSREEMTKNQVSLTCLVKGFYPSDIAVEWESNGQPENNYKTTPPVLDSDGSFFLYSKLTVDKSRWQQGNVFSCSVMHEALHNHYTQKSLSLSPGK

SEQ ID NO: 32 - DNA, 1152 bp, Artificial Sequence
  Description of Artificial Sequence: Synthetic polynucleotide
atggatgcaatgaagagagggctctgctgtgtgctgctgctgtgtggagcagtcttcgtttcgcccggcgcccagaagtcggttaataacgacatgatagtcactgacaacaacggtgcagtcaagtttccacaactgtgtaaattttgtgatgtgagattttccacctgtgacaaccagaaatcctgcatgagcaactgcagcatcacctccatctgtgagaagccacaggaagtctgtgtggctgtatggagaaagaatgacgagaacataacactagagacagtttgccatgaccccaagctcccctaccatgactttattctggaagatgctgcttctccaaagtgcattatgaaggaaaaaaaaaagcctggtgagactttcttcatgtgttcctgtagctctgatgagtgcaatgacaacatcatcttctcagaagaatataacaccagcaatcctgacaccggtggtggaactcacacatgcccaccgtgcccagcacctgaactcctggggggaccgtcagtcttcctcttccccccaaaacccaaggacaccctcatgatctcccggacccctgaggtcacatgcgtggtggtggacgtgagccacgaagaccctgaggtcaagttcaactggtacgtggacggcgtggaggtgcataatgccaagacaaagccgcgggaggagcagtacaacagcacgtaccgtgtggtcagcgtcctcaccgtcctgcaccaggactggctgaatggcaaggagtacaagtgcaaggtctccaacaaagccctcccagcccccatcgagaaaaccatctccaaagccaaagggcagccccgagaaccacaggtgtacaccctgcccccatcccgggaggagatgaccaagaaccaggtcagcctgacctgcctggtcaaaggcttctatcccagcgacatcgccgtggagtgggagagcaatgggcagccggagaacaactacaagaccacgcctcccgtgctggactccgacggctccttcttcctctatagcaagctcaccgtggacaagagcaggtggcagcaggggaacgtcttctcatgctccgtgatgcatgaggctctgcacaaccactacacgcagaagagcctctccctgtccccgggtaaa

SEQ ID NO: 33 - protein, 376 aa, Artificial Sequence
  Description of Artificial Sequence: Synthetic polypeptide
MDAMKRGLCCVLLLCGAVFVSPGADMIVTDNNGAVKFPQLCKFCDVRFSTCDNQKSCMSNCSITSICEKPQEVCVAVWRKNDENITLETVCHDPKLPYHDFILEDAASPKCIMKEKKKPGETFFMCSCSSDECNDNIIFSEEYNTSNPDTGGGVECPPCPAPPVAGPSVFLFPPKPKDTLMISRTPEVTCVVVDVSHEDPEVQFNWYVDGVEVHNAKTKPREEQFNSTFRVVSVLTVVHQDWLNGKEYKCKVSNKGLPAPIEKTISKTKGQPREPQVYTLPPSREEMTKNQVSLTCLVKGFYPSDIAVEWESNGQPENNYKTTPPMLDSDGSFFLYSKLTVDKSRWQQGNVFSCSVMHEALHNHYTQKSLSLSPGK

SEQ ID NO: 34 - DNA, 1128 bp, Artificial Sequence
  Description of Artificial Sequence: Synthetic polynucleotide
atggatgcaatgaagagagggctctgctgtgtgctgctgctgtgtggagcagtcttcgtttcgcccggcgccgacatgatagtcactgacaacaacggtgcagtcaagtttccacaactgtgtaaattttgtgatgtgagattttccacctgtgacaaccagaaatcctgcatgagcaactgcagcatcacctccatctgtgagaagccacaggaagtctgtgtggctgtatggagaaagaatgacgagaacataacactagagacagtttgccatgaccccaagctcccctaccatgactttattctggaagatgctgcttctccaaagtgcattatgaaggaaaaaaaaaagcctggtgagactttcttcatgtgttcctgtagctctgatgagtgcaatgacaacatcatcttctcagaagaatataacaccagcaatcctgacaccggtggtggagtcgagtgcccaccgtgcccagcaccacctgtggcaggaccgtcagtcttcctcttccccccaaaacccaaggacaccctcatgatctcccggacccctgaggtcacgtgcgtggtggtggacgtgagccacgaagaccccgaggtccagttcaactggtacgtggacggcgtggaggtgcataatgccaagacaaagccacgggaggagcagttcaacagcacgttccgtgtggtcagcgtcctcaccgtcgtgcaccaggactggctgaacggcaaggagtacaagtgcaaggtctccaacaaaggcctcccagcccccatcgagaaaaccatctccaaaaccaaagggcagccccgagaaccacaggtgtacaccctgcccccatcccgggaggagatgaccaagaaccaggtcagcctgacctgcctggtcaaaggcttctaccccagcgacatcgccgtggagtgggagagcaatgggcagccggagaacaactacaagaccacacctcccatgctggactccgacggctccttcttcctctacagcaagctcaccgtggacaagagcaggtggcagcaggggaacgtcttctcatgctccgtgatgcatgaggctctgcacaaccactacacgcagaagagcctctccctgtctccgggtaaa

SEQ ID NO: 35 - protein, 378 aa, Artificial Sequence
  Description of Artificial Sequence: Synthetic polypeptide
MDAMKRGLCCVLLLCGAVFVSPGADMIVTDNNGAVKFPQLCKFCDVRFSTCDNQKSCMSNCSITSICEKPQEVCVAVWRKNDENITLETVCHDPKLPYHDFILEDAASPKCIMKEKKKPGETFFMCSCSSDECNDNIIFSEEYNTSNPDTGGGTHTCPPCPAPELLGGPSVFLFPPKPKDTLMISRTPEVTCVVVDVSHEDPEVKFNWYVDGVEVHNAKTKPREEQYNSTYRVVSVLTVLHQDWLNGKEYKCKVSNKALPAPIEKTISKAKGQPREPQVYTLPPSREEMTKNQVSLTCLVKGFYPSDIAVEWESNGQPENNYKTTPPVLDSDGSFFLYSKLTVDKSRWQQGNVFSCSVMHEALHNHYTQKSLSLSPGK

SEQ ID NO: 36 - DNA, 1134 bp, Artificial Sequence
  Description of Artificial Sequence: Synthetic polynucleotide
atggatgcaatgaagagagggctctgctgtgtgctgctgctgtgtggagcagtcttcgtttcgcccggcgccgacatgatagtcactgacaacaacggtgcagtcaagtttccacaactgtgtaaattttgtgatgtgagattttccacctgtgacaaccagaaatcctgcatgagcaactgcagcatcacctccatctgtgagaagccacaggaagtctgtgtggctgtatggagaaagaatgacgagaacataacactagagacagtttgccatgaccccaagctcccctaccatgactttattctggaagatgctgcttctccaaagtgcattatgaaggaaaaaaaaaagcctggtgagactttcttcatgtgttcctgtagctctgatgagtgcaatgacaacatcatcttctcagaagaatataacaccagcaatcctgacaccggtggtggaactcacacatgcccaccgtgcccagcacctgaactcctggggggaccgtcagtcttcctcttccccccaaaacccaaggacaccctcatgatctcccggacccctgaggtcacatgcgtggtggtggacgtgagccacgaagaccctgaggtcaagttcaactggtacgtggacggcgtggaggtgcataatgccaagacaaagccgcgggaggagcagtacaacagcacgtaccgtgtggtcagcgtcctcaccgtcctgcaccaggactggctgaatggcaaggagtacaagtgcaaggtctccaacaaagccctcccagcccccatcgagaaaaccatctccaaagccaaagggcagccccgagaaccacaggtgtacaccctgcccccatcccgggaggagatgaccaagaaccaggtcagcctgacctgcctggtcaaaggcttctatcccagcgacatcgccgtggagtgggagagcaatgggcagccggagaacaactacaagaccacgcctcccgtgctggactccgacggctccttcttcctctatagcaagctcaccgtggacaagagcaggtggcagcaggggaacgtcttctcatgctccgtgatgcatgaggctctgcacaaccactacacgcagaagagcctctccctgtccccgggtaaa

SEQ ID NO: 37 - protein, 382 aa, Artificial Sequence
  Description of Artificial Sequence: Synthetic polypeptide
MDAMKRGLCCVLLLCGAVFVSPGATIPPHVQKSVNNDMIVTDNNGAVKFPQLCKFCDVRFSTCDNQKSCMSNCSITSICEKPQEVCVAVWRKNDENITLETVCHDPKLPYHDFILEDAASPKCIMKEKKKPGETFFMCSCSSDECNDNIIFSEEYTGGGVECPPCPAPPVAGPSVFLFPPKPKDTLMISRTPEVTCVVVDVSHEDPEVQFNWYVDGVEVHNAKTKPREEQFNSTFRVVSVLTVVHQDWLNGKEYKCKVSNKGLPAPIEKTISKTKGQPREPQVYTLPPSREEMTKNQVSLTCLVKGFYPSDIAVEWESNGQPENNYKTTPPMLDSDGSFFLYSKLTVDKSRWQQGNVFSCSVMHEALHNHYTQKSLSLSPGK

SEQ ID NO: 38 - DNA, 1146 bp, Artificial Sequence
  Description of Artificial Sequence: Synthetic polynucleotide
atggatgcaatgaagagagggctctgctgtgtgctgctgctgtgtggagcagtcttcgtttcgcccggcgccacgatcccaccgcacgttcagaagtcggttaataacgacatgatagtcactgacaacaacggtgcagtcaagtttccacaactgtgtaaattttgtgatgtgagattttccacctgtgacaaccagaaatcctgcatgagcaactgcagcatcacctccatctgtgagaagccacaggaagtctgtgtggctgtatggagaaagaatgacgagaacataacactagagacagtttgccatgaccccaagctcccctaccatgactttattctggaagatgctgcttctccaaagtgcattatgaaggaaaaaaaaaagcctggtgagactttcttcatgtgttcctgtagctctgatgagtgcaatgacaacatcatcttctcagaagaatataccggtggtggagtcgagtgcccaccgtgcccagcaccacctgtggcaggaccgtcagtcttcctcttccccccaaaacccaaggacaccctcatgatctcccggacccctgaggtcacgtgcgtggtggtggacgtgagccacgaagaccccgaggtccagttcaactggtacgtggacggcgtggaggtgcataatgccaagacaaagccacgggaggagcagttcaacagcacgttccgtgtggtcagcgtcctcaccgtcgtgcaccaggactggctgaacggcaaggagtacaagtgcaaggtctccaacaaaggcctcccagcccccatcgagaaaaccatctccaaaaccaaagggcagccccgagaaccacaggtgtacaccctgcccccatcccgggaggagatgaccaagaaccaggtcagcctgacctgcctggtcaaaggcttctaccccagcgacatcgccgtggagtgggagagcaatgggcagccggagaacaactacaagaccacacctcccatgctggactccgacggctccttcttcctctacagcaagctcaccgtggacaagagcaggtggcagcaggggaacgtcttctcatgctccgtgatgcatgaggctctgcacaaccactacacgcagaagagcctctccctgtctccgggtaaa

SEQ ID NO: 39 - protein, 384 aa, Artificial Sequence
  Description of Artificial Sequence: Synthetic polypeptide
MDAMKRGLCCVLLLCGAVFVSPGATIPPHVQKSVNNDMIVTDNNGAVKFPQLCKFCDVRFSTCDNQKSCMSNCSITSICEKPQEVCVAVWRKNDENITLETVCHDPKLPYHDFILEDAASPKCIMKEKKKPGETFFMCSCSSDECNDNIIFSEEYTGGGTHTCPPCPAPELLGGPSVFLFPPKPKDTLMISRTPEVTCVVVDVSHEDPEVKFNWYVDGVEVHNAKTKPREEQYNSTYRVVSVLTVLHQDWLNGKEYKCKVSNKALPAPIEKTISKAKGQPREPQVYTLPPSREEMTKNQVSLTCLVKGFYPSDIAVEWESNGQPENNYKTTPPVLDSDGSFFLYSKLTVDKSRWQQGNVFSCSVMHEALHNHYTQKSLSLSPGK

SEQ ID NO: 40 - DNA, 1152 bp, Artificial Sequence
  Description of Artificial Sequence: Synthetic polynucleotide
atggatgcaatgaagagagggctctgctgtgtgctgctgctgtgtggagcagtcttcgtttcgcccggcgccacgatcccaccgcacgttcagaagtcggttaataacgacatgatagtcactgacaacaacggtgcagtcaagtttccacaactgtgtaaattttgtgatgtgagattttccacctgtgacaaccagaaatcctgcatgagcaactgcagcatcacctccatctgtgagaagccacaggaagtctgtgtggctgtatggagaaagaatgacgagaacataacactagagacagtttgccatgaccccaagctcccctaccatgactttattctggaagatgctgcttctccaaagtgcattatgaaggaaaaaaaaaagcctggtgagactttcttcatgtgttcctgtagctctgatgagtgcaatgacaacatcatcttctcagaagaatataccggtggtggaactcacacatgcccaccgtgcccagcacctgaactcctggggggaccgtcagtcttcctcttccccccaaaacccaaggacaccctcatgatctcccggacccctgaggtcacatgcgtggtggtggacgtgagccacgaagaccctgaggtcaagttcaactggtacgtggacggcgtggaggtgcataatgccaagacaaagccgcgggaggagcagtacaacagcacgtaccgtgtggtcagcgtcctcaccgtcctgcaccaggactggctgaatggcaaggagtacaagtgcaaggtctccaacaaagccctcccagcccccatcgagaaaaccatctccaaagccaaagggcagccccgagaaccacaggtgtacaccctgcccccatcccgggaggagatgaccaagaaccaggtcagcctgacctgcctggtcaaaggcttctatcccagcgacatcgccgtggagtgggagagcaatgggcagccggagaacaactacaagaccacgcctcccgtgctggactccgacggctccttcttcctctatagcaagctcaccgtggacaagagcaggtggcagcaggggaacgtcttctcatgctccgtgatgcatgaggctctgcacaaccactacacgcagaagagcctctccctgtccccgggtaaa

SEQ ID NO: 41 - protein, 382 aa, Artificial Sequence
  Description of Artificial Sequence: Synthetic polypeptide
MDAMKRGLCCVLLLCGAVFVSPGATIPPHVQKSVNNDMIVTDNNGAVKFPQLCKFCDVRFSTCDNQKSCMSDCSITSICEKPQEVCVAVWRKNDENITLETVCHDPKLPYHDFILEDAASPKCIMKEKKKPGETFFMCSCSSDECNDNIIFSEEYTGGGVECPPCPAPPVAGPSVFLFPPKPKDTLMISRTPEVTCVVVDVSHEDPEVQFNWYVDGVEVHNAKTKPREEQFNSTFRVVSVLTVVHQDWLNGKEYKCKVSNKGLPAPIEKTISKTKGQPREPQVYTLPPSREEMTKNQVSLTCLVKGFYPSDIAVEWESNGQPENNYKTTPPMLDSDGSFFLYSKLTVDKSRWQQGNVFSCSVMHEALHNHYTQKSLSLSPGK

SEQ ID NO: 42 - DNA, 1146 bp, Artificial Sequence
  Description of Artificial Sequence: Synthetic polynucleotide
atggatgcaatgaagagagggctctgctgtgtgctgctgctgtgtggagcagtcttcgtttcgcccggcgccacgatcccaccgcacgttcagaagtcggttaataacgacatgatagtcactgacaacaacggtgcagtcaagtttccacaactgtgtaaattttgtgatgtgagattttccacctgtgacaaccagaaatcctgcatgagcgactgcagcatcacctccatctgtgagaagccacaggaagtctgtgtggctgtatggagaaagaatgacgagaacataacactagagacagtttgccatgaccccaagctcccctaccatgactttattctggaagatgctgcttctccaaagtgcattatgaaggaaaaaaaaaagcctggtgagactttcttcatgtgttcctgtagctctgatgagtgcaatgacaacatcatcttctcagaagaatataccggtggtggagtcgagtgcccaccgtgcccagcaccacctgtggcaggaccgtcagtcttcctcttccccccaaaacccaaggacaccctcatgatctcccggacccctgaggtcacgtgcgtggtggtggacgtgagccacgaagaccccgaggtccagttcaactggtacgtggacggcgtggaggtgcataatgccaagacaaagccacgggaggagcagttcaacagcacgttccgtgtggtcagcgtcctcaccgtcgtgcaccaggactggctgaacggcaaggagtacaagtgcaaggtctccaacaaaggcctcccagcccccatcgagaaaaccatctccaaaaccaaagggcagccccgagaaccacaggtgtacaccctgcccccatcccgggaggagatgaccaagaaccaggtcagcctgacctgcctggtcaaaggcttctaccccagcgacatcgccgtggagtgggagagcaatgggcagccggagaacaactacaagaccacacctcccatgctggactccgacggctccttcttcctctacagcaagctcaccgtggacaagagcaggtggcagcaggggaacgtcttctcatgctccgtgatgcatgaggctctgcacaaccactacacgcagaagagcctctccctgtctccgggtaaa

SEQ ID NO: 43 - protein, 384 aa, Artificial Sequence
  Description of Artificial Sequence: Synthetic polypeptide
MDAMKRGLCCVLLLCGAVFVSPGATIPPHVQKSVNNDMIVTDNNGAVKFPQLCKFCDVRFSTCDNQKSCMSDCSITSICEKPQEVCVAVWRKNDENITLETVCHDPKLPYHDFILEDAASPKCIMKEKKKPGETFFMCSCSSDECNDNIIFSEEYTGGGTHTCPPCPAPELLGGPSVFLFPPKPKDTLMISRTPEVTCVVVDVSHEDPEVKFNWYVDGVEVHNAKTKPREEQYNSTYRVVSVLTVLHQDWLNGKEYKCKVSNKALPAPIEKTISKAKGQPREPQVYTLPPSREEMTKNQVSLTCLVKGFYPSDIAVEWESNGQPENNYKTTPPVLDSDGSFFLYSKLTVDKSRWQQGNVFSCSVMHEALHNHYTQKSLSLSPGK

SEQ ID NO: 44 - DNA, 1152 bp, Artificial Sequence
  Description of Artificial Sequence: Synthetic polynucleotide
atggatgcaatgaagagagggctctgctgtgtgctgctgctgtgtggagcagtcttcgtttcgcccggcgccacgatcccaccgcacgttcagaagtcggttaataacgacatgatagtcactgacaacaacggtgcagtcaagtttccacaactgtgtaaattttgtgatgtgagattttccacctgtgacaaccagaaatcctgcatgagcgactgcagcatcacctccatctgtgagaagccacaggaagtctgtgtggctgtatggagaaagaatgacgagaacataacactagagacagtttgccatgaccccaagctcccctaccatgactttattctggaagatgctgcttctccaaagtgcattatgaaggaaaaaaaaaagcctggtgagactttcttcatgtgttcctgtagctctgatgagtgcaatgacaacatcatcttctcagaagaatataccggtggtggaactcacacatgcccaccgtgcccagcacctgaactcctggggggaccgtcagtcttcctcttccccccaaaacccaaggacaccctcatgatctcccggacccctgaggtcacatgcgtggtggtggacgtgagccacgaagaccctgaggtcaagttcaactggtacgtggacggcgtggaggtgcataatgccaagacaaagccgcgggaggagcagtacaacagcacgtaccgtgtggtcagcgtcctcaccgtcctgcaccaggactggctgaatggcaaggagtacaagtgcaaggtctccaacaaagccctcccagcccccatcgagaaaaccatctccaaagccaaagggcagccccgagaaccacaggtgtacaccctgcccccatcccgggaggagatgaccaagaaccaggtcagcctgacctgcctggtcaaaggcttctatcccagcgacatcgccgtggagtgggagagcaatgggcagccggagaacaactacaagaccacgcctcccgtgctggactccgacggctccttcttcctctatagcaagctcaccgtggacaagagcaggtggcagcaggggaacgtcttctcatgctccgtgatgcatgaggctctgcacaaccactacacgcagaagagcctctccctgtccccgggtaaa

SEQ ID NO: 45 - protein, 35 aa, Homo sapiens
QKSDVEMEAQKDEIICPSCNRTAHPLRHINNDMIV

SEQ ID NO: 46 - protein, 4 aa, Homo sapiens
DMIV

SEQ ID NO: 47 - protein, 119 aa, Artificial Sequence
  Description of Artificial Sequence: Synthetic polypeptide
DMIVTDNNGAVKFPQLCKFCDVRFSTCDNQKSCMSNCSITSICEKPQEVCVAVWRKNDENITLETVCHDPKLPYHDFILEDAASPKCIMKEKKKPGETFFMCSCSSDECNDNIIFSEEY

SEQ ID NO: 48 - protein, 125 aa, Artificial Sequence
  Description of Artificial Sequence: Synthetic polypeptide
QKSVNNDMIVTDNNGAVKFPQLCKFCDVRFSTCDNQKSCMSNCSITSICEKPQEVCVAVWRKNDENITLETVCHDPKLPYHDFILEDAASPKCIMKEKKKPGETFFMCSCSSDECNDNIIFSEEY

SEQ ID NO: 49 - protein, 150 aa, Artificial Sequence
  Description of Artificial Sequence: Synthetic polypeptide
QKSDVEMEAQKDEIICPSCNRTAHPLRHINNDMIVTDNNGAVKFPQLCKFCDVRFSTCDNQKSCMSNCSITSICEKPQEVCVAVWRKNDENITLETVCHDPKLPYHDFILEDAASPKCIMKEKKKPGETFFMCSCSSDECNDNIIFSEEY

SEQ ID NO: 50 - protein, 364 aa, Artificial Sequence
  Description of Artificial Sequence: Synthetic polypeptide
TIPPHVQKSVNNDMIVTDNNGAVKFPQLCKFCDVRFSTCDNQKSCMSNCSITSICEKPQEVCVAVWRKNDENITLETVCHDPKLPYHDFILEDAASPKCIMKEKKKPGETFFMCSCSSDECNDNIIFSEEYNTSNPDTGGGVECPPCPAPPVAGPSVFLFPPKPKDTLMISRTPEVTCVVVDVSHEDPEVQFNWYVDGVEVHNAKTKPREEQFNSTFRVVSVLTVVHQDWLNGKEYKCKVSNKGLPAPIEKTISKTKGQPREPQVYTLPPSREEMTKNQVSLTCLVKGFYPSDIAVEWESNGQPENNYKTTPPMLDSDGSFFLYSKLTVDKSRWQQGNVFSCSVMHEALHNHYTQKSLSLSPGK

SEQ ID NO: 51 - DNA, 1164 bp, Artificial Sequence
  Description of Artificial Sequence: Synthetic polynucleotide
atggatgcaatgaagagagggctctgctgtgtgctgctgctgtgtggagcagtcttcgtttcgcccggcgccacgatcccaccgcacgttcagaagtcggttaataacgacatgatagtcactgacaacaacggtgcagtcaagtttccacaactgtgtaaattttgtgatgtgagattttccacctgtgacaaccagaaatcctgcatgagcaactgcagcatcacctccatctgtgagaagccacaggaagtctgtgtggctgtatggagaaagaatgacgagaacataacactagagacagtttgccatgaccccaagctcccctaccatgactttattctggaagatgctgcttctccaaagtgcattatgaaggaaaaaaaaaagcctggtgagactttcttcatgtgttcctgtagctctgatgagtgcaatgacaacatcatcttctcagaagaatataacaccagcaatcctgacaccggtggtggagtcgagtgcccaccgtgcccagcaccacctgtggcaggaccgtcagtcttcctcttccccccaaaacccaaggacaccctcatgatctcccggacccctgaggtcacgtgcgtggtggtggacgtgagccacgaagaccccgaggtccagttcaactggtacgtggacggcgtggaggtgcataatgccaagacaaagccacgggaggagcagttcaacagcacgttccgtgtggtcagcgtcctcaccgtcgtgcaccaggactggctgaacggcaaggagtacaagtgcaaggtctccaacaaaggcctcccagcccccatcgagaaaaccatctccaaaaccaaagggcagccccgagaaccacaggtgtacaccctgcccccatcccgggaggagatgaccaagaaccaggtcagcctgacctgcctggtcaaaggcttctaccccagcgacatcgccgtggagtgggagagcaatgggcagccggagaacaactacaagaccacacctcccatgctggactccgacggctccttcttcctctacagcaagctcaccgtggacaagagcaggtggcagcaggggaacgtcttctcatgctccgtgatgcatgaggctctgcacaaccactacacgcagaagagcctctccctgtctccgggtaaa

SEQ ID NO: 52 - protein, 388 aa, Artificial Sequence
  Description of Artificial Sequence: Synthetic polypeptide
MDAMKRGLCCVLLLCGAVFVSPGATIPPHVQKSVNNDMIVTDNNGAVKFPQLCKFCDVRFSTCDNQKSCMSNCSITSICEKPQEVCVAVWRKNDENITLETVCHDPKLPYHDFILEDAASPKCIMKEKKKPGETFFMCSCSSDECNDNIIFSEEYNTSNPDTGGGVECPPCPAPPVAGPSVFLFPPKPKDTLMISRTPEVTCVVVDVSHEDPEVQFNWYVDGVEVHNAKTKPREEQFNSTFRVVSVLTVVHQDWLNGKEYKCKVSNKGLPAPIEKTISKTKGQPREPQVYTLPPSREEMTKNQVSLTCLVKGFYPSDIAVEWESNGQPENNYKTTPPMLDSDGSFFLYSKLTVDKSRWQQGNVFSCSVMHEALHNHYTQKSLSLSPGK

SEQ ID NO: 53 - protein, 364 aa, Artificial Sequence
  Description of Artificial Sequence: Synthetic polypeptide
TIPPHVQKSVNNDMIVTDNNGAVKFPQLCKFCDVRFSTCDNQKSCMSNCSITSICEKPQEVCVAVWRKNDENITLETVCHDPKLPYHKFILEDAASPKCIMKEKKKPGETFFMCSCSSDECNDNIIFSEEYNTSNPDTGGGVECPPCPAPPVAGPSVFLFPPKPKDTLMISRTPEVTCVVVDVSHEDPEVQFNWYVDGVEVHNAKTKPREEQFNSTFRVVSVLTVVHQDWLNGKEYKCKVSNKGLPAPIEKTISKTKGQPREPQVYTLPPSREEMTKNQVSLTCLVKGFYPSDIAVEWESNGQPENNYKTTPPMLDSDGSFFLYSKLTVDKSRWQQGNVFSCSVMHEALHNHYTQKSLSLSPGK

SEQ ID NO: 54 - protein, 366 aa, Artificial Sequence
  Description of Artificial Sequence: Synthetic polypeptide
TIPPHVQKSVNNDMIVTDNNGAVKFPQLCKFCDVRFSTCDNQKSCMSNCSITSICEKPQEVCVAVWRKNDENITLETVCHDPKLPYHKFILEDAASPKCIMKEKKKPGETFFMCSCSSDECNDNIIFSEEYNTSNPDTGGGTHTCPPCPAPELLGGPSVFLFPPKPKDTLMISRTPEVTCVVVDVSHEDPEVKFNWYVDGVEVHNAKTKPREEQYNSTYRVVSVLTVLHQDWLNGKEYKCKVSNKALPAPIEKTISKAKGQPREPQVYTLPPSREEMTKNQVSLTCLVKGFYPSDIAVEWESNGQPENNYKTTPPVLDSDGSFFLYSKLTVDKSRWQQGNVFSCSVMHEALHNHYTQKSLSLSPGK

SEQ ID NO: 55 - protein, 358 aa, Artificial Sequence
  Description of Artificial Sequence: Synthetic polypeptide
QKSVNNDMIVTDNNGAVKFPQLCKFCDVRFSTCDNQKSCMSNCSITSICEKPQEVCVAVWRKNDENITLETVCHDPKLPYHDFILEDAASPKCIMKEKKKPGETFFMCSCSSDECNDNIIFSEEYNTSNPDTGGGVECPPCPAPPVAGPSVFLFPPKPKDTLMISRTPEVTCVVVDVSHEDPEVQFNWYVDGVEVHNAKTKPREEQFNSTFRVVSVLTVVHQDWLNGKEYKCKVSNKGLPAPIEKTISKTKGQPREPQVYTLPPSREEMTKNQVSLTCLVKGFYPSDIAVEWESNGQPENNYKTTPPMLDSDGSFFLYSKLTVDKSRWQQGNVFSCSVMHEALHNHYTQKSLSLSPGK

SEQ ID NO: 56 - protein, 360 aa, Artificial Sequence
  Description of Artificial Sequence: Synthetic polypeptide
QKSVNNDMIVTDNNGAVKFPQLCKFCDVRFSTCDNQKSCMSNCSITSICEKPQEVCVAVWRKNDENITLETVCHDPKLPYHDFILEDAASPKCIMKEKKKPGETFFMCSCSSDECNDNIIFSEEYNTSNPDTGGGTHTCPPCPAPELLGGPSVFLFPPKPKDTLMISRTPEVTCVVVDVSHEDPEVKFNWYVDGVEVHNAKTKPREEQYNSTYRVVSVLTVLHQDWLNGKEYKCKVSNKALPAPIEKTISKAKGQPREPQVYTLPPSREEMTKNQVSLTCLVKGFYPSDIAVEWESNGQPENNYKTTPPVLDSDGSFFLYSKLTVDKSRWQQGNVFSCSVMHEALHNHYTQKSLSLSPGK

SEQ ID NO: 57 - protein, 352 aa, Artificial Sequence
  Description of Artificial Sequence: Synthetic polypeptide
DMIVTDNNGAVKFPQLCKFCDVRFSTCDNQKSCMSNCSITSICEKPQEVCVAVWRKNDENITLETVCHDPKLPYHDFILEDAASPKCIMKEKKKPGETFFMCSCSSDECNDNIIFSEEYNTSNPDTGGGVECPPCPAPPVAGPSVFLFPPKPKDTLMISRTPEVTCVVVDVSHEDPEVQFNWYVDGVEVHNAKTKPREEQFNSTFRVVSVLTVVHQDWLNGKEYKCKVSNKGLPAPIEKTISKTKGQPREPQVYTLPPSREEMTKNQVSLTCLVKGFYPSDIAVEWESNGQPENNYKTTPPMLDSDGSFFLYSKLTVDKSRWQQGNVFSCSVMHEALHNHYTQKSLSLSPGK

SEQ ID NO: 58 - protein, 354 aa, Artificial Sequence
  Description of Artificial Sequence: Synthetic polypeptide
DMIVTDNNGAVKFPQLCKFCDVRFSTCDNQKSCMSNCSITSICEKPQEVCVAVWRKNDENITLETVCHDPKLPYHDFILEDAASPKCIMKEKKKPGETFFMCSCSSDECNDNIIFSEEYNTSNPDTGGGTHTCPPCPAPELLGGPSVFLFPPKPKDTLMISRTPEVTCVVVDVSHEDPEVKFNWYVDGVEVHNAKTKPREEQYNSTYRVVSVLTVLHQDWLNGKEYKCKVSNKALPAPIEKTISKAKGQPREPQVYTLPPSREEMTKNQVSLTCLVKGFYPSDIAVEWESNGQPENNYKTTPPVLDSDGSFFLYSKLTVDKSRWQQGNVFSCSVMHEALHNHYTQKSLSLSPGK

SEQ ID NO: 59 - protein, 358 aa, Artificial Sequence
  Description of Artificial Sequence: Synthetic polypeptide
TIPPHVQKSVNNDMIVTDNNGAVKFPQLCKFCDVRFSTCDNQKSCMSNCSITSICEKPQEVCVAVWRKNDENITLETVCHDPKLPYHDFILEDAASPKCIMKEKKKPGETFFMCSCSSDECNDNIIFSEEYTGGGVECPPCPAPPVAGPSVFLFPPKPKDTLMISRTPEVTCVVVDVSHEDPEVQFNWYVDGVEVHNAKTKPREEQFNSTFRVVSVLTVVHQDWLNGKEYKCKVSNKGLPAPIEKTISKTKGQPREPQVYTLPPSREEMTKNQVSLTCLVKGFYPSDIAVEWESNGQPENNYKTTPPMLDSDGSFFLYSKLTVDKSRWQQGNVFSCSVMHEALHNHYTQKSLSLSPGK

SEQ ID NO: 60 - protein, 360 aa, Artificial Sequence
  Description of Artificial Sequence: Synthetic polypeptide
TIPPHVQKSVNNDMIVTDNNGAVKFPQLCKFCDVRFSTCDNQKSCMSNCSITSICEKPQEVCVAVWRKNDENITLETVCHDPKLPYHDFILEDAASPKCIMKEKKKPGETFFMCSCSSDECNDNIIFSEEYTGGGTHTCPPCPAPELLGGPSVFLFPPKPKDTLMISRTPEVTCVVVDVSHEDPEVKFNWYVDGVEVHNAKTKPREEQYNSTYRVVSVLTVLHQDWLNGKEYKCKVSNKALPAPIEKTISKAKGQPREPQVYTLPPSREEMTKNQVSLTCLVKGFYPSDIAVEWESNGQPENNYKTTPPVLDSDGSFFLYSKLTVDKSRWQQGNVFSCSVMHEALHNHYTQKSLSLSPGK

SEQ ID NO: 61 - protein, 358 aa, Artificial Sequence
  Description of Artificial Sequence: Synthetic polypeptide
TIPPHVQKSVNNDMIVTDNNGAVKFPQLCKFCDVRFSTCDNQKSCMSDCSITSICEKPQEVCVAVWRKNDENITLETVCHDPKLPYHDFILEDAASPKCIMKEKKKPGETFFMCSCSSDECNDNIIFSEEYTGGGVECPPCPAPPVAGPSVFLFPPKPKDTLMISRTPEVTCVVVDVSHEDPEVQFNWYVDGVEVHNAKTKPREEQFNSTFRVVSVLTVVHQDWLNGKEYKCKVSNKGLPAPIEKTISKTKGQPREPQVYTLPPSREEMTKNQVSLTCLVKGFYPSDIAVEWESNGQPENNYKTTPPMLDSDGSFFLYSKLTVDKSRWQQGNVFSCSVMHEALHNHYTQKSLSLSPGK

SEQ ID NO: 62 - protein, 360 aa, Artificial Sequence
  Description of Artificial Sequence: Synthetic polypeptide
TIPPHVQKSVNNDMIVTDNNGAVKFPQLCKFCDVRFSTCDNQKSCMSDCSITSICEKPQEVCVAVWRKNDENITLETVCHDPKLPYHDFILEDAASPKCIMKEKKKPGETFFMCSCSSDECNDNIIFSEEYTGGGTHTCPPCPAPELLGGPSVFLFPPKPKDTLMISRTPEVTCVVVDVSHEDPEVKFNWYVDGVEVHNAKTKPREEQYNSTYRVVSVLTVLHQDWLNGKEYKCKVSNKALPAPIEKTISKAKGQPREPQVYTLPPSREEMTKNQVSLTCLVKGFYPSDIAVEWESNGQPENNYKTTPPVLDSDGSFFLYSKLTVDKSRWQQGNVFSCSVMHEALHNHYTQKSLSLSPGK

SEQ ID NO: 63 - protein, 6 aa, Artificial Sequence
  Description of Artificial Sequence: Synthetic 6xHis tag
HHHHHH

SEQ ID NO: 64 - protein, 38 aa, Homo sapiens
MGRGLLRGLWPLHIVLWTRIASTIPPHVQKSVNNDMIV

SEQ ID NO: 65 - protein, 16 aa, Homo sapiens
TIPPHVQKSVNNDMIV

SEQ ID NO: 66 - protein, 10 aa, Homo sapiens
QKSVNNDMIV

SEQ ID NO: 67 - protein, 4 aa, Homo sapiens
DMIV

SEQ ID NO: 68 - protein, 63 aa, Homo sapiens
MGRGLLRGLWPLHIVLWTRIASTIPPHVQKSDVEMEAQKDEIICPSCNRTAHPLRHINNDMIV

SEQ ID NO: 69 - protein, 41 aa, Homo sapiens
TIPPHVQKSDVEMEAQKDEIICPSCNRTAHPLRHINNDMIV